European Patent Application EP 4 471 131 A1, published December 4, 2024. Title: 一种流感病毒的致弱方法及流感致弱病毒株和应用. Applicant: 浙江迪福润丝生物科技有限公司. The sequence listing filed with the application follows.

SEQUENCE LISTING (21 sequences)

SEQ ID NO: 1 - DNA, 280 bp, 人工序列(Artificial Sequence)
atgagtcttctaaccgaggtcgaaacgcctatcagaaacgaatgggggtgcagatgcaacggttcaagtgatcgcaaatatcattgggatcttgcacttgacattgtggattcttgatcgtctttttttcaaatgcatttaccgtcgctttaaatacggactgaaaggagggccttctacggaaggagtgccaaagtctatgagggaagaatatcgaaaggaacagcagagtgctgtggatgctgacgatggtcattttgtcagcatagagctggagtaa

SEQ ID NO: 2 - DNA, 274 bp, 人工序列(Artificial Sequence)
atgagtcttctaaccgaggtcgaaacgcctatcagaaacgaatgggggtgcagatgcaacggttcaagtgatcctctcactattgctgcacttgacattgtggattcttgatcgtctttttttcaaatgcatttaccgtcgctttaaatacggactgaaaggagggccttctacggaaggagtgccaaagtctatgagggaagaatatcgaaaggaacagcagagtgctgtggatgctgacgatggtcattttgtcagcatagagctggagtaa

SEQ ID NO: 3 - DNA, 272 bp, 人工序列(Artificial Sequence)
atgagtcttctaaccgaggtcgaaacgcctatcagaaacgaatgggggtgcagatgcaacggttcaagtgatcctctcactattgccgcaaatatcattgggatcttgcacttgacattgtggattctttttaccgtcgctttaaatacggactgaaaggagggccttctacggaaggagtgccaaagtctatgagggaagaatatcgaaaggaacagcagagtgctgtggatgctgacgatggtcattttgtcagcatagagctggagtaa

SEQ ID NO: 4 - DNA, 256 bp, 人工序列(Artificial Sequence)
atgagtcttctaaccgaggtcgaaacgcctatcagaaacgaatgggggtgcagatgcaacggttcaagtgatcctctcactattgccgcaaatatcattgggatcttgcacttgacattgtggattcttgatcgtctttttttcaaatgcatctacggaaggagtgccaaagtctatgagggaagaatatcgaaaggaacagcagagtgctgtggatgctgacgatggtcattttgtcagcatagagctggagtaa

SEQ ID NO: 5 - DNA, 229 bp, 人工序列(Artificial Sequence)
atgagtcttctaaccgaggtcgaaacgcctatcagaaacgaatgggggtgcagatgcaacggttcaagtgatcctctcactattgctttaccgtcgctttaaatacggactgaaaggagggccttctacggaaggagtgccaaagtctatgagggaagaatatcgaaaggaacagcagagtgctgtggatgctgacgatggtcattttgtcagcatagagctggagtaa

SEQ ID NO: 6 - DNA, 191 bp, 人工序列(Artificial Sequence)
atgagtcttctaaccgaggtcgaaacgcctatcagaaacgaatgggggtgcagatgcaacggttcaagtgatcctctcactattgctctacggaaggagtgccaaagtctatgagggaagaatatcgaaaggaacagcagagtgctgtggatgctgacgatggtcattttgtcagcatagagctggagtaa

SEQ ID NO: 7 - DNA, 294 bp, 人工序列(Artificial Sequence)
atgagtcttctaaccgaggtcgaaacgcctatcagaaacgaatgggggtgcagatgcaacggttcaagtgatcctctcactattgccgcaaatatcattgggatcttgcacttgacattgtggattcttgatcgtctttttttcaaatgcatttaccgtcgctttaaatacggactgaaaggagggccttctacggaaggagtgccaaagtctatgagggaagaatatcgaaaggaacagcagagtgctgtggatgctgacgatggtcattttgtcagcatagagctggagtaa

SEQ ID NO: 8 - DNA, 37 bp, 人工序列(Artificial Sequence)
aacggttcaagtgatcgcaaatatcattgggatcttg

SEQ ID NO: 9 - DNA, 22 bp, 人工序列(Artificial Sequence)
atcacttgaaccgttgcatctg

SEQ ID NO: 10 - DNA, 39 bp, 人工序列(Artificial Sequence)
tcctctcactattgctgcacttgacattgtggattcttg

SEQ ID NO: 11 - DNA, 22 bp, 人工序列(Artificial Sequence)
gcaatagtgagaggatcacttg

SEQ ID NO: 12 - DNA, 36 bp, 人工序列(Artificial Sequence)
acattgtggattctttttaccgtcgctttaaatacg

SEQ ID NO: 13 - DNA, 21 bp, 人工序列(Artificial Sequence)
aagaatccacaatgtcaagtg

SEQ ID NO: 14 - DNA, 36 bp, 人工序列(Artificial Sequence)
tttttttcaaatgcatctacggaaggagtgccaaag

SEQ ID NO: 15 - DNA, 19 bp, 人工序列(Artificial Sequence)
tgcatttgaaaaaaagacg

SEQ ID NO: 16 - DNA, 36 bp, 人工序列(Artificial Sequence)
tcctctcactattgctttaccgtcgctttaaatacg

SEQ ID NO: 17 - DNA, 22 bp, 人工序列(Artificial Sequence)
gcaatagtgagaggatcacttg

SEQ ID NO: 18 - DNA, 36 bp, 人工序列(Artificial Sequence)
tcctctcactattgctctacggaaggagtgccaaag

SEQ ID NO: 19 - DNA, 22 bp, 人工序列(Artificial Sequence)
gcaatagtgagaggatcacttg

SEQ ID NO: 20 - DNA, 31 bp, 人工序列(Artificial Sequence)
cacacacgtctccgggagcaaaagcaggtag

SEQ ID NO: 21 - DNA, 38 bp, 人工序列(Artificial Sequence)
cacacacgtctcctattagtagaaacaaggtagttttt